European Patent Specification EP 4 162 046 B1, published October 16, 2024. Title: Treatment method of left ventricular dysfunction following an acute myocardial infarction. Applicant: Universidad de Murcia. Application PCT. The sequence listing filed with the application follows.

SEQUENCE LISTING (68 sequences)

SEQ ID NO: 1 - RNA, 21 nt, Artificial Sequence
  siRNA (1) sense sequence
cuguuguccagaauacuuauu

SEQ ID NO: 2 - RNA, 21 nt, Artificial Sequence
  siRNA (1) antisense sequence
uaaguauucuggacaacaguu

SEQ ID NO: 3 - RNA, 21 nt, Artificial Sequence
  siRNA (2) sense sequence
cauguagaaucaaauauuauu

SEQ ID NO: 4 - RNA, 21 nt, Artificial Sequence
  siRNA (2) antisense sequence
uaauauuugauucuacauguu

SEQ ID NO: 5 - RNA, 21 nt, Artificial Sequence
  siRNA (3) sense sequence
gcuccaagaacaauagcuuuu

SEQ ID NO: 6 - RNA, 21 nt, Artificial Sequence
  siRNA (3) antisense sequence
aagcuauuguucuuggagcuu

SEQ ID NO: 7 - RNA, 21 nt, Artificial Sequence
  siRNA (4) sense sequence
caacuaaccugaaaucucauu

SEQ ID NO: 8 - RNA, 21 nt, Artificial Sequence
  siRNA (4) antisense sequence
ugagauuucagguuaguuguu

SEQ ID NO: 9 - RNA, 21 nt, Artificial Sequence
  non-targeting Accell siRNA sense sequences (siCtrl)
uagcgacuaaacacaucaauu

SEQ ID NO: 10 - RNA, 21 nt, Artificial Sequence
  non-targeting Accell siRNA antisense sequences (siCtrl)
uugauguguuuagucgcuauu

SEQ ID NO: 11 - DNA, 20 bp, Artificial Sequence
  BNP-F
cgtcttggccttttggcttc

SEQ ID NO: 12 - DNA, 23 bp, Artificial Sequence
  BNP-R
ggtggtctagcaggttcttgaaa

SEQ ID NO: 13 - DNA, 19 bp, Artificial Sequence
  Col1a1-F
ctggcaagaagggagatga

SEQ ID NO: 14 - DNA, 20 bp, Artificial Sequence
  Col1a1-R
caccatccaaaccactgaaa

SEQ ID NO: 15 - DNA, 24 bp, Artificial Sequence
  Col3a1-F
acagcaaattcacttacacagttc

SEQ ID NO: 16 - DNA, 19 bp, Artificial Sequence
  Col3a1-R
ctcattgccttgcgtgttt

SEQ ID NO: 17 - DNA, 25 bp, Artificial Sequence
  CRP-F
gaactttcagccgaatacatctttt

SEQ ID NO: 18 - DNA, 21 bp, Artificial Sequence
  CRP-R
ccttcctcgacatgtctgtct

SEQ ID NO: 19 - DNA, 22 bp, Artificial Sequence
  IL-33-F
cagaatcatcgagaaaaggcgg

SEQ ID NO: 20 - DNA, 20 bp, Artificial Sequence
  IL-33-R
gccggggaaatcttggagtt

SEQ ID NO: 21 - DNA, 20 bp, Artificial Sequence
  IL-6-F
cacttcacaagtcggaggct

SEQ ID NO: 22 - DNA, 22 bp, Artificial Sequence
  IL-6-R
tgccattgcacaactcttttct

SEQ ID NO: 23 - DNA, 20 bp, Artificial Sequence
  Myh6-F
accaacctgtccaagttccg

SEQ ID NO: 24 - DNA, 20 bp, Artificial Sequence
  Myh6-R
gtcgtgcatcttcttggcac

SEQ ID NO: 25 - DNA, 20 bp, Artificial Sequence
  Myh7-F
cgcatcaaggagctcaccta

SEQ ID NO: 26 - DNA, 20 bp, Artificial Sequence
  Myh7-R
cttggacaggttggtgttgg

SEQ ID NO: 27 - DNA, 22 bp, Artificial Sequence
  MyO-F
catggttgcaccgtgctcacag

SEQ ID NO: 28 - DNA, 20 bp, Artificial Sequence
  MyO-R
gagcccatggctcagccctg

SEQ ID NO: 29 - DNA, 20 bp, Artificial Sequence
  Nppa-F
gcttccaggccatattggag

SEQ ID NO: 30 - DNA, 19 bp, Artificial Sequence
  Nppa-R
gggggcatgacctcatctt

SEQ ID NO: 31 - DNA, 21 bp, Artificial Sequence
  PTX3-F
caggatgcacgcttccaaaaa

SEQ ID NO: 32 - DNA, 19 bp, Artificial Sequence
  PTX3-R
tgcccgcaggttgtgaaac

SEQ ID NO: 33 - DNA, 22 bp, Artificial Sequence
  Smad2-F
aagccatcaccactcagaattg

SEQ ID NO: 34 - DNA, 23 bp, Artificial Sequence
  Smad2-R
cactgatctaccgtatttgctgt

SEQ ID NO: 35 - DNA, 21 bp, Artificial Sequence
  Smad3-F
gaggagaagtggtgcgagaag

SEQ ID NO: 36 - DNA, 21 bp, Artificial Sequence
  Smad3-R
atgcacttggtgttcacgttc

SEQ ID NO: 37 - DNA, 24 bp, Artificial Sequence
  sST2-F
gctaggacctctggctaatgtatc

SEQ ID NO: 38 - DNA, 20 bp, Artificial Sequence
  sST2-R
atggtgtgttcactaggcgg

SEQ ID NO: 39 - DNA, 20 bp, Artificial Sequence
  ST2L-F
tgggcaaggtaaaccgactg

SEQ ID NO: 40 - DNA, 20 bp, Artificial Sequence
  ST2L-R
caccccctcctcactaccta

SEQ ID NO: 41 - DNA, 20 bp, Artificial Sequence
  TGF-b-F
caacccaggtccttcctaaa

SEQ ID NO: 42 - DNA, 20 bp, Artificial Sequence
  TGF-b-R
ggagagccctggataccaac

SEQ ID NO: 43 - DNA, 20 bp, Artificial Sequence
  TNF-a-F
agttctatggcccagaccct

SEQ ID NO: 44 - DNA, 19 bp, Artificial Sequence
  TNF-a-R
ggtggtttgctacgacgtg

SEQ ID NO: 45 - DNA, 20 bp, Artificial Sequence
  Yy1-F
tgagaaagcatctgcacacc

SEQ ID NO: 46 - DNA, 20 bp, Artificial Sequence
  Yy1-R
cgcaaattgaagtccagtga

SEQ ID NO: 47 - DNA, 23 bp, Artificial Sequence
  a-SMA-F
gtgctgtccctctatgcctctgg

SEQ ID NO: 48 - DNA, 23 bp, Artificial Sequence
  a-SMA-R
ggcacgttgtgagtcacaccatc

SEQ ID NO: 49 - RNA, 19 nt, Artificial Sequence
  siRNA 5 sense sequence
cauguaguaucaaauauua

SEQ ID NO: 50 - RNA, 19 nt, Artificial Sequence
  siRNA 5 antisense sequence
uaauauuugauacuacaug

SEQ ID NO: 51 - RNA, 19 nt, Artificial Sequence
  siRNA 6 sense sequence
gggauaugcuuaguaaugc

SEQ ID NO: 52 - RNA, 19 nt, Artificial Sequence
  siRNA 6 antisense sequence
uaauauuugauacuacaug

SEQ ID NO: 53 - RNA, 19 nt, Artificial Sequence
  siRNA 7 sense sequence
cucaguuguagaauguauu

SEQ ID NO: 54 - RNA, 19 nt, Artificial Sequence
  siRNA 7 antisense sequence
uaauauuugauacuacaug

SEQ ID NO: 55 - RNA, 19 nt, Artificial Sequence
  siRNA 8 sense sequence
caacuaaccugaaaucuca

SEQ ID NO: 56 - RNA, 19 nt, Artificial Sequence
  siRNA 8 antisense sequence
uaauauuugauacuacaug

SEQ ID NO: 57 - DNA, 19 bp, Artificial Sequence
  GAPDH-F
gtgaaggtcggtgtgaacg

SEQ ID NO: 58 - DNA, 20 bp, Artificial Sequence
  GAPDH-R
tcgttgatggcaacaatctc

SEQ ID NO: 59 - DNA, 24 bp, Artificial Sequence
  GAPDH-F
tcaacgaccactttgtcaagctca

SEQ ID NO: 60 - DNA, 23 bp, Artificial Sequence
  GAPDH-R
gctggtggtccaggggtcttact

SEQ ID NO: 61 - DNA, 21 bp, Artificial Sequence
  Myh6-F
caagccaacaccaacctgtcc

SEQ ID NO: 62 - DNA, 20 bp, Artificial Sequence
  Myh6-R
ttggcaagagtgaggttccc

SEQ ID NO: 63 - DNA, 21 bp, Artificial Sequence
  Myh7-F
ctcgccagaatggagtacaaa

SEQ ID NO: 64 - DNA, 20 bp, Artificial Sequence
  Myh7-R
cttcatccagggccaattct

SEQ ID NO: 65 - DNA, 20 bp, Artificial Sequence
  Nppa-F
ccccggttcagcctcggact

SEQ ID NO: 66 - DNA, 20 bp, Artificial Sequence
  Nppa-R
acggatgccctcggtggcta

SEQ ID NO: 67 - DNA, 19 bp, Artificial Sequence
  Yy1-F
acatctgcacacccacggt

SEQ ID NO: 68 - DNA, 19 bp, Artificial Sequence
  Yy1-R
gcgtttcccacagccttcg